European Patent Application EP 4 785 946 A1, published August 5, 2026. Title: 一种脂质修饰的核酸化合物、其制备方法及用途. Applicant: 上海拓界生物医药科技有限公司. Application WO. The sequence listing filed with the application follows.

SEQUENCE LISTING (48 sequences)

SEQ ID NO: 1 - RNA, 21 nt, synthetic construct
  source 1..21: mol_type = other RNA
  modified_base 1..5: mod_base = OTHER; note = modified with 2'-methoxy; note (original language) = 2'甲氧基修饰
  modified_base 6: mod_base = OTHER; note = modified with 2'-Fluoro; note (original language) = 2'-氟修饰
  modified_base 7: mod_base = OTHER; note = modified with 2'-methoxy; note (original language) = 2‘甲氧基修饰
  modified_base 8..10: mod_base = OTHER; note = modified with 2'-Fluoro; note (original language) = 2'-氟修饰
  modified_base 11..21: mod_base = OTHER; note = modified with 2'-methoxy; note (original language) = 2'-甲氧基修饰
  modified_base 1..3: mod_base = OTHER; note = two adjacent nucleosides are linked by phosphorothioate diester groups; note (original language) = 相邻的两个核苷之间通过硫代磷酸二酯基连接
  modified_base 19..21: mod_base = OTHER; note = two adjacent nucleosides are linked by phosphorothioate diester groups; note (original language) = 相邻的两个核苷之间通过硫代磷酸二酯基连接
  modified_base 21: mod_base = OTHER; note = conjugated to A01''; note (original language) = 和A01''缀合
ccggtcccaggttatgacaca

SEQ ID NO: 2 - RNA, 23 nt, synthetic construct
  source 1..23: mol_type = other RNA
  modified_base 1: mod_base = OTHER; note = 5'-E-VP; note (original language) = 5'末端为反式-乙烯基磷酸二酯基
  modified_base 2: mod_base = OTHER; note = mofied with 2'-Fluoro; note (original language) = 2'-F修饰
  modified_base 6: mod_base = OTHER; note = modified with 2'-Fluoro; note (original language) = 2'-氟修饰
  modified_base 8..9: mod_base = OTHER; note = modified with 2'-Fluoro; note (original language) = 2'-氟修饰
  modified_base 14: mod_base = OTHER; note = modified with 2'-Fluoro; note (original language) = 2'-氟修饰
  modified_base 16: mod_base = OTHER; note = modified with 2'-Fluoro; note (original language) = 2'-氟修饰
  modified_base 1: mod_base = OTHER; note = modified with 2'-methoxy; note (original language) = 2'-甲氧基修饰
  modified_base 3..5: mod_base = OTHER; note = modified with 2'-methoxy; note (original language) = 2'-甲氧基修饰
  modified_base 7: mod_base = OTHER; note = modified with 2'-methoxy; note (original language) = 2'-甲氧基修饰
  modified_base 10..13: mod_base = OTHER; note = modified with 2'-methoxy; note (original language) = 2'-甲氧基修饰
  modified_base 15: mod_base = OTHER; note = modified with 2'-methoxy; note (original language) = 2'-甲氧基修饰
  modified_base 17..23: mod_base = OTHER; note = modified with 2'-methoxy; note (original language) = 2'-甲氧基修饰
  modified_base 1..3: mod_base = OTHER; note = two adjacent nucleosides are linked by phosphorothioate diester groups; note (original language) = 相邻的两个核苷之间通过硫代磷酸二酯基连接
  modified_base 21..23: mod_base = OTHER; note = two adjacent nucleosides are linked by phosphorothioate diester groups; note (original language) = 相邻的两个核苷之间沟通过硫代磷酸二酯基连接
tgtgtcataacctgggaccggat

SEQ ID NO: 3 - RNA, 21 nt, Synthetic construct
  source 1..21: mol_type = other RNA
  modified_base 1..3: mod_base = OTHER; note = two adjacentnucleosides a linked by phosphorothioate diestei groups; note (original language) = 相邻的两个核苷之间通过硫代磷酸二酯基连接
  modified_base 7: mod_base = OTHER; note = modified with 2'-methoxy; note (original language) = 2'-甲氧基修饰
  modified_base 8..10: mod_base = OTHER; note = modified with 2'-Fluoro; note (original language) = 2'-氟修饰
  modified_base 6: mod_base = OTHER; note = modified with 2'-Fluoro; note (original language) = 2'-氟修饰
  modified_base 11..21: mod_base = OTHER; note = modified with 2'-methoxy; note (original language) = 2'-甲氧基修饰
  modified_base 19..21: mod_base = OTHER; note = two adjacentnucleosides a linked by phosphorothioate diestei groups; note (original language) = 相邻的两个核苷之间通过硫代磷酸二酯基连接
  modified_base 1..5: mod_base = OTHER; note = modified with 2'-methoxy; note (original language) = 2'-甲氧基修饰
  modified_base 21: mod_base = OTHER; note = conjugated to A02''; note (original language) = 和A02''缀合
ccggtcccaggttatgacaca

SEQ ID NO: 4 - RNA, 21 nt, synthetic construct
  source 1..21: mol_type = other RNA
  modified_base 1..3: mod_base = OTHER; note = two adjacentnucleosides a linked by phosphorothioate diestei groups; note (original language) = 相邻的两个核苷之间通过硫代磷酸二酯基连接
  modified_base 7: mod_base = OTHER; note = modified with 2'-methoxy; note (original language) = 2'-甲氧基修饰
  modified_base 8..10: mod_base = OTHER; note = modified with 2'-Fluoro; note (original language) = 2'-氟修饰
  modified_base 6: mod_base = OTHER; note = modified with 2'-Fluoro; note (original language) = 2'-氟修饰
  modified_base 11..21: mod_base = OTHER; note = modified with 2'-methoxy; note (original language) = 2'-甲氧基修饰
  modified_base 19..21: mod_base = OTHER; note = =two adjacentnucleosides a linked by phosphorothioate diestei groups; note (original language) = 相邻的两个核苷之间通过硫代磷酸二酯基连接
  modified_base 1..5: mod_base = OTHER; note = modified with 2'-methoxy; note (original language) = 2'-甲氧基修饰
  modified_base 21: mod_base = OTHER; note = conjugated to A03''; note (original language) = 和A03''缀合
ccggtcccaggttatgacaca

SEQ ID NO: 5 - RNA, 21 nt, synthetic construct
  source 1..21: mol_type = other RNA
  modified_base 1..3: mod_base = OTHER; note = two adjacentnucleosides a linked by phosphorothioate diestei groups; note (original language) = 相邻的两个核苷之间通过硫代磷酸二酯基连接
  modified_base 7: mod_base = OTHER; note = modified with 2'-methoxy; note (original language) = 2'-甲氧基修饰
  modified_base 8..10: mod_base = OTHER; note = modified with 2'-Fluoro; note (original language) = 2'-氟修饰
  modified_base 6: mod_base = OTHER; note = modified with 2'-Fluoro; note (original language) = 2'-氟修饰
  modified_base 11..21: mod_base = OTHER; note = modified with 2'-methoxy; note (original language) = 2'-甲氧基修饰
  modified_base 19..21: mod_base = OTHER; note = two adjacentnucleosides a linked by phosphorothioate diestei groups; note (original language) = 相邻的两个核苷之间通过硫代磷酸二酯基连接
  modified_base 1..5: mod_base = OTHER; note = modified with 2'-methoxy; note (original language) = 2'-甲氧基修饰
  modified_base 1: mod_base = OTHER; note = conjugated to A04''; note (original language) = 和A04''缀合
ccggtcccaggttatgacaca

SEQ ID NO: 6 - RNA, 21 nt, synthetic construct
  source 1..21: mol_type = other RNA
  modified_base 1..3: mod_base = OTHER; note = two adjacentnucleosides a linked by phosphorothioate diestei groups; note (original language) = 相邻的两个核苷之间通过硫代磷酸二酯基连接
  modified_base 7: mod_base = OTHER; note = modified with 2'-methoxy; note (original language) = 2'-甲氧基修饰
  modified_base 8..10: mod_base = OTHER; note = modified with 2'-Fluoro; note (original language) = 2'-氟修饰
  modified_base 6: mod_base = OTHER; note = modified with 2'-Fluoro; note (original language) = 2'-氟修饰
  modified_base 11..21: mod_base = OTHER; note = modified with 2'-methoxy; note (original language) = 2'-甲氧基修饰
  modified_base 19..21: mod_base = OTHER; note = two adjacentnucleosides a linked by phosphorothioate diestei groups; note (original language) = 相邻的两个核苷之间通过硫代磷酸二酯基连接
  modified_base 1..5: mod_base = OTHER; note = modified with 2'-methoxy; note (original language) = 2'-甲氧基修饰
  modified_base 1: mod_base = OTHER; note = conjugated to A05''; note (original language) = 和A05‘'缀合
ccggtcccaggttatgacaca

SEQ ID NO: 7 - RNA, 21 nt, synthetic construct
  source 1..21: mol_type = other RNA
  modified_base 1..3: mod_base = OTHER; note = two adjacentnucleosides a linked by phosphorothioate diestei groups; note (original language) = 相邻的两个核苷之间通过硫代磷酸二酯基连接
  modified_base 7: mod_base = OTHER; note = modified with 2'-methoxy; note (original language) = 2'-甲氧基修饰
  modified_base 8..10: mod_base = OTHER; note = modified with 2'-Fluoro; note (original language) = 2'-氟修饰
  modified_base 6: mod_base = OTHER; note = modified with 2'-Fluoro; note (original language) = 2'-氟修饰
  modified_base 11..21: mod_base = OTHER; note = modified with 2'-methoxy; note (original language) = 2'-甲氧基修饰
  modified_base 19..21: mod_base = OTHER; note = two adjacentnucleosides a linked by phosphorothioate diestei groups; note (original language) = 相邻的两个核苷之间通过硫代磷酸二酯基连接
  modified_base 1..5: mod_base = OTHER; note = modified with 2'-methoxy; note (original language) = 2'-甲氧基修饰
  modified_base 21: mod_base = OTHER; note = conjugated to A06''; note (original language) = 和A06''缀合
ccggtcccaggttatgacaca

SEQ ID NO: 8 - RNA, 21 nt, synthetic construct
  source 1..21: mol_type = other RNA
  modified_base 9..11: mod_base = OTHER; note = modified with 2'-Fluoro; note (original language) = 2'-氟修饰
  modified_base 1..8: mod_base = OTHER; note = modified with 2'-methoxy; note (original language) = 2'-甲氧基修饰
  modified_base 12..21: mod_base = OTHER; note = modified with 2'-methoxy; note (original language) = 2'-甲氧基修饰
  modified_base 1..3: mod_base = OTHER; note = two adjacentnucleosides a linked by phosphorothioate diestei groups; note (original language) = 相邻的两个核苷之间通过硫代磷酸二酯基连接
  modified_base 19..21: mod_base = OTHER; note = two adjacentnucleosides a linked by phosphorothioate diestei groups; note (original language) = 相邻的两个核苷之间通过硫代磷酸二酯基连接
  modified_base 21: mod_base = OTHER; note = conjugated to A01''; note (original language) = 和A01''缀合
ttcactttatcaatagttcca

SEQ ID NO: 9 - RNA, 23 nt, synthetic construct
  source 1..23: mol_type = other RNA
  modified_base 1: mod_base = OTHER; note = 5'-E-VP; note (original language) = 5'末端为反式-乙烯基磷酸二酯基
  modified_base 2: mod_base = OTHER; note = modified with 2'-Fluoro; note (original language) = 2'-氟修饰
  modified_base 6: mod_base = OTHER; note = modified with 2'-Fluoro; note (original language) = 2'-氟修饰
  modified_base 12: mod_base = OTHER; note = modified with 2'-Fluoro; note (original language) = 2'-氟修饰
  modified_base 14: mod_base = OTHER; note = modified with 2'-Fluoro; note (original language) = 2'-氟修饰
  modified_base 16: mod_base = OTHER; note = modified with 2'-Fluoro; note (original language) = 2'-氟修饰
  modified_base 1: mod_base = OTHER; note = modified with 2'-methoxy; note (original language) = 2'-甲氧基修饰
  modified_base 3..5: mod_base = OTHER; note = modified with 2'-methoxy; note (original language) = 2'-甲氧基修饰
  modified_base 7..11: mod_base = OTHER; note = modified with 2'-methoxy; note (original language) = 2'-甲氧基修饰
  modified_base 13: mod_base = OTHER; note = modified with 2'-methoxy; note (original language) = 2'-甲氧基修饰
  modified_base 14: mod_base = OTHER; note = modified with 2'-methoxy; note (original language) = 2'-甲氧基修饰
  modified_base 17..23: mod_base = OTHER; note = modified with 2'-methoxy; note (original language) = 2'-甲氧基修饰
  modified_base 1..3: mod_base = OTHER; note = =two adjacentnucleosides a linked by phosphorothioate diestei groups; note (original language) = 相邻的两个核苷之间通过硫代磷酸二酯基连接
  modified_base 21..23: mod_base = OTHER; note = two adjacentnucleosides a linked by phosphorothioate diestei groups; note (original language) = 相邻的两个核苷之间通过硫代磷酸二酯基连接
tggaactattgataaagtgaatt

SEQ ID NO: 10 - RNA, 21 nt, synthetic construct
  source 1..21: mol_type = other RNA
  modified_base 1..3: mod_base = OTHER; note = two adjacentnucleosides a linked by phosphorothioate diestei groups; note (original language) = 相邻的两个核苷之间通过硫代磷酸二酯基连接
  modified_base 9..11: mod_base = OTHER; note = modified with 2'-Fluoro; note (original language) = 2'-氟修饰
  modified_base 1..8: mod_base = OTHER; note = modified with 2'-methoxy; note (original language) = 2'-甲氧基修饰
  modified_base 12..21: mod_base = OTHER; note = modified with 2'-methoxy; note (original language) = 2‘-甲氧基修饰
  modified_base 19..21: mod_base = OTHER; note = two adiacentnucleosides a linked by phosphorothioate diestei groups; note (original language) = 相邻的两个核苷之间通过硫代磷酸二酯基连接
  modified_base 21: mod_base = OTHER; note = conjugated to A02''; note (original language) = 和A02''缀合
ttcactttatcaatagttcca

SEQ ID NO: 11 - RNA, 21 nt, synthetic construct
  source 1..21: mol_type = other RNA
  modified_base 9..11: mod_base = OTHER; note = modified with 2'-Fluoro; note (original language) = 2'-氟修饰
  modified_base 1..8: mod_base = OTHER; note = modified with 2'-methoxy; note (original language) = 2'-甲氧基修饰
  modified_base 12..21: mod_base = OTHER; note = modified with 2'-methoxy; note (original language) = 2'-甲氧基修饰
  modified_base 1..3: mod_base = OTHER; note = two adiacentnucleosides a linked by phosphorothioate diestei groups; note (original language) = 相邻的两个核苷之间通过硫代磷酸二酯基连接
  modified_base 19..21: mod_base = OTHER; note = two adiacentnucleosides a linked by phosphorothioate diestei groups; note (original language) = 相邻的两个核苷之间通过硫代磷酸二酯基连接
  modified_base 21: mod_base = OTHER; note = conjugated to A03''; note (original language) = 和A03''缀合
ttcactttatcaatagttcca

SEQ ID NO: 12 - RNA, 21 nt, synthetic construct
  source 1..21: mol_type = other RNA
  modified_base 9..11: mod_base = OTHER; note = modified with 2'-Fluoro; note (original language) = 2'-氟修饰
  modified_base 1..8: mod_base = OTHER; note = modified with 2'-methoxy; note (original language) = 2'-甲氧基修饰
  modified_base 12..21: mod_base = OTHER; note = modified with 2'-methoxy; note (original language) = 2'-甲氧基修饰
  modified_base 1..3: mod_base = OTHER; note = two adiacentnucleosides a linked by phosphorothioate diestei groups; note (original language) = 相邻的两个核苷之间通过硫代磷酸二酯基连接
  modified_base 19..21: mod_base = OTHER; note = two adiacentnucleosides a linked by phosphorothioate diestei groups; note (original language) = 相邻的两个核苷之间通过硫代磷酸二酯基连接
  modified_base 1: mod_base = OTHER; note = conjugated to A04''; note (original language) = 和A04''缀合
ttcactttatcaatagttcca

SEQ ID NO: 13 - RNA, 21 nt, synthetic construct
  source 1..21: mol_type = other RNA
  modified_base 9..11: mod_base = OTHER; note = modified with 2'-Fluoro; note (original language) = 2'-氟修饰
  modified_base 1..8: mod_base = OTHER; note = modified with 2'-methoxy; note (original language) = 2'-甲氧基修饰
  modified_base 12..21: mod_base = OTHER; note = modified with 2'-methoxy; note (original language) = 2'-甲氧基修饰
  modified_base 1..3: mod_base = OTHER; note = two adiacentnucleosides a linked by phosphorothioate diestei groups; note (original language) = 相邻的两个核苷之间通过硫代磷酸二酯基连接
  modified_base 19..21: mod_base = OTHER; note = two adiacentnucleosides a linked by phosphorothioate diestei groups; note (original language) = 相邻的两个核苷之间通过硫代磷酸二酯基连接
  modified_base 1: mod_base = OTHER; note = conjugated to A05''; note (original language) = 和A05''缀合
ttcactttatcaatagttcca

SEQ ID NO: 14 - RNA, 21 nt, synthetic construct
  source 1..21: mol_type = other RNA
  modified_base 9..11: mod_base = OTHER; note = modified with 2'-Fluoro; note (original language) = 2'-氟修饰
  modified_base 1..8: mod_base = OTHER; note = modified with 2'-methoxy; note (original language) = 2'-甲氧基修饰
  modified_base 12..21: mod_base = OTHER; note = modified with 2'-methoxy; note (original language) = 2'-甲氧基修饰
  modified_base 1..3: mod_base = OTHER; note = two adiacentnucleosides a linked by phosphorothioate diestei groups; note (original language) = 相邻的两个核苷之间通过硫代磷酸二酯基连接
  modified_base 19..21: mod_base = OTHER; note = two adiacentnucleosides a linked by phosphorothioate diestei groups; note (original language) = 相邻的两个核苷之间通过硫代磷酸二酯基连接
  modified_base 21: mod_base = OTHER; note = conjugated to A06''; note (original language) = 和A06''缀合
ttcactttatcaatagttcca

SEQ ID NO: 15 - RNA, 21 nt, synthetic construct
  source 1..21: mol_type = other RNA
  modified_base 9..11: mod_base = OTHER; note = modified with 2'-Fluoro; note (original language) = 2'-氟修饰
  modified_base 1..8: mod_base = OTHER; note = modified with 2'-methoxy; note (original language) = 2'-甲氧基修饰
  modified_base 12..21: mod_base = OTHER; note = modified with 2'-methoxy; note (original language) = 2'-甲氧基修饰
  modified_base 1..3: mod_base = OTHER; note = two adiacentnucleosides a linked by phosphorothioate diestei groups; note (original language) = 相邻的两个核苷之间通过硫代磷酸二酯基连接
  modified_base 19..21: mod_base = OTHER; note = two adiacentnucleosides a linked by phosphorothioate diestei groups; note (original language) = 相邻的两个核苷之间通过硫代磷酸二酯基连接
  modified_base 21: mod_base = OTHER; note = conjugated to A01''; note (original language) = 和A01''缀合
ttcgccaactattctacgtga

SEQ ID NO: 16 - RNA, 23 nt, synthetic construct
  source 1..23: mol_type = other RNA
  modified_base 2: mod_base = OTHER; note = modified with 2'-Fluoro; note (original language) = 2'-氟修饰
  modified_base 4: mod_base = OTHER; note = modified with 2'-Fluoro; note (original language) = 2'-氟修饰
  modified_base 6: mod_base = OTHER; note = modified with 2'-Fluoro; note (original language) = 2'-氟修饰
  modified_base 10: mod_base = OTHER; note = modified with 2'-Fluoro; note (original language) = 2'-氟修饰
  modified_base 12: mod_base = OTHER; note = modified with 2'-Fluoro; note (original language) = 2'-氟修饰
  modified_base 14: mod_base = OTHER; note = modified with 2'-Fluoro; note (original language) = 2'-氟修饰
  modified_base 16: mod_base = OTHER; note = modified with 2'-Fluoro; note (original language) = 2'-氟修饰
  modified_base 18: mod_base = OTHER; note = modified with 2'-Fluoro; note (original language) = 2'-氟修饰
  modified_base 1: mod_base = OTHER; note = modified with 2'-methoxy; note (original language) = 2'-甲氧基修饰
  modified_base 3: mod_base = OTHER; note = modified with 2'-methoxy; note (original language) = 2'-甲氧基修饰
  modified_base 5: mod_base = OTHER; note = modified with 2'-methoxy; note (original language) = 2'-甲氧基修饰
  modified_base 7..9: mod_base = OTHER; note = modified with 2'-methoxy; note (original language) = 2'-甲氧基修饰
  modified_base 11: mod_base = OTHER; note = modified with 2'-methoxy; note (original language) = 2'-甲氧基修饰
  modified_base 13: mod_base = OTHER; note = modified with 2'-methoxy; note (original language) = 2'-甲氧基修饰
  modified_base 15: mod_base = OTHER; note = modified with 2'-methoxy; note (original language) = 2'-甲氧基修饰
  modified_base 17: mod_base = OTHER; note = modified with 2'-methoxy; note (original language) = 2'-甲氧基修饰
  modified_base 19..23: mod_base = OTHER; note = modified with 2'-methoxy; note (original language) = 2'-甲氧基修饰
  modified_base 1: mod_base = OTHER; note = 5'-E-VP; note (original language) = 5'末端为反式-乙烯基磷酸二酯基
  modified_base 1..3: mod_base = OTHER; note = two adiacentnucleosides a linked by phosphorothioate diestei groups; note (original language) = 相邻的两个核苷之间通过硫代磷酸二酯基连接
  modified_base 21..23: mod_base = OTHER; note = two adiacentnucleosides a linked by phosphorothioate diestei groups; note (original language) = 相邻的两个核苷之间通过硫代磷酸二酯基连接
tcacgtagaatagttgccgaagg

SEQ ID NO: 17 - RNA, 21 nt, synthetic construct
  source 1..21: mol_type = other RNA
  modified_base 9..11: mod_base = OTHER; note = modified with 2'-Fluoro; note (original language) = 2'-氟修饰
  modified_base 1..8: mod_base = OTHER; note = modified with 2'-methoxy; note (original language) = 2'-甲氧基修饰
  modified_base 12..21: mod_base = OTHER; note = modified with 2'-methoxy; note (original language) = 2'-甲氧基修饰
  modified_base 1..3: mod_base = OTHER; note = two adiacentnucleosides a linked by phosphorothioate diestei groups; note (original language) = 相邻的两个核苷之间通过硫代磷酸二酯基连接
  modified_base 19..21: mod_base = OTHER; note = two adiacentnucleosides a linked by phosphorothioate diestei groups; note (original language) = 相邻的两个核苷之间通过硫代磷酸二酯基连接
  modified_base 21: mod_base = OTHER; note = conjugated to A02''; note (original language) = 和A02''缀合
ttcgccaactattctacgtga

SEQ ID NO: 18 - RNA, 21 nt, synthetic construct
  source 1..21: mol_type = other RNA
  modified_base 9..11: mod_base = OTHER; note = modified with 2'-Fluoro; note (original language) = 2'-氟修饰
  modified_base 1..8: mod_base = OTHER; note = modified with 2'-methoxy; note (original language) = 2'-甲氧基修饰
  modified_base 12..21: mod_base = OTHER; note = modified with 2'-methoxy; note (original language) = 2'-甲氧基
  modified_base 1..3: mod_base = OTHER; note = two adiacentnucleosides a linked by phosphorothioate diestei groups; note (original language) = 相邻的两个核苷之间通过硫代磷酸二酯基连接
  modified_base 19..21: mod_base = OTHER; note = two adiacentnucleosides a linked by phosphorothioate diestei groups; note (original language) = 相邻的两个核苷之间通过硫代磷酸二酯基连接
  modified_base 21: mod_base = OTHER; note = conjugated to A03''; note (original language) = 和A03''缀合
ttcgccaactattctacgtga

SEQ ID NO: 19 - RNA, 21 nt, synthetic construct
  source 1..21: mol_type = other RNA
  modified_base 9..11: mod_base = OTHER; note = modified with 2'-Fluoro; note (original language) = 2‘-氟修饰
  modified_base 1..8: mod_base = OTHER; note = modified with 2'-methoxy; note (original language) = 2'-甲氧基修饰
  modified_base 12..21: mod_base = OTHER; note = modified with 2'-methoxy; note (original language) = 2'-甲氧基修饰
  modified_base 1..3: mod_base = OTHER; note = two adiacentnucleosides a linked by phosphorothioate diestei groups; note (original language) = 相邻的两个核苷之间通过硫代磷酸二酯基连接
  modified_base 19..21: mod_base = OTHER; note = two adiacentnucleosides a linked by phosphorothioate diestei groups; note (original language) = 相邻的两个核苷之间通过硫代磷酸二酯基连接
  modified_base 1: mod_base = OTHER; note = conjugated to A04''; note (original language) = 和A04''缀合
ttcgccaactattctacgtga

SEQ ID NO: 20 - RNA, 21 nt, synthetic construct
  source 1..21: mol_type = other RNA
  modified_base 9..11: mod_base = OTHER; note = modified with 2'-Fluoro; note (original language) = 2'-氟修饰
  modified_base 1..8: mod_base = OTHER; note = modified with 2'-methoxy; note (original language) = 2'-甲氧基修饰
  modified_base 12..21: mod_base = OTHER; note = modified with 2'-methoxy; note (original language) = 2'-甲氧基修饰
  modified_base 1..3: mod_base = OTHER; note = two adiacentnucleosides a linked by phosphorothioate diestei groups; note (original language) = 相邻的两个核苷之间通过硫代磷酸二酯基连接
  modified_base 19..21: mod_base = OTHER; note = two adiacentnucleosides a linked by phosphorothioate diestei groups; note (original language) = 相邻的两个核苷之间通过硫代磷酸二酯基连接
  modified_base 1: mod_base = OTHER; note = conjugated to A05''; note (original language) = 和A05''缀合
ttcgccaactattctacgtga

SEQ ID NO: 21 - RNA, 21 nt, synthetic construct
  source 1..21: mol_type = other RNA
  modified_base 9..11: mod_base = OTHER; note = modified with 2'-Fluoro; note (original language) = 2'-氟修饰
  modified_base 1..8: mod_base = OTHER; note = modified with 2'-methoxy; note (original language) = 2'-甲氧基修饰
  modified_base 12..21: mod_base = OTHER; note = modified with 2'-methoxy; note (original language) = 2'-甲氧基修饰
  modified_base 1..3: mod_base = OTHER; note = two adiacentnucleosides a linked by phosphorothioate diestei groups; note (original language) = 相邻的两个核苷之间通过硫代磷酸二酯基连接
  modified_base 19..21: mod_base = OTHER; note = two adiacentnucleosides a linked by phosphorothioate diestei groups; note (original language) = 相邻的两个核苷之间通过硫代磷酸二酯基连接
  modified_base 21: mod_base = OTHER; note = conjugated to A06''; note (original language) = 和A06''缀合
ttcgccaactattctacgtga

SEQ ID NO: 22 - RNA, 21 nt, synthetic construct
  source 1..21: mol_type = other RNA
  modified_base 9..11: mod_base = OTHER; note = modified with 2'-Fluoro; note (original language) = 2'-氟修饰
  modified_base 1..8: mod_base = OTHER; note = modified with 2'-methoxy; note (original language) = 2'-甲氧基修饰
  modified_base 12..21: mod_base = OTHER; note = modified with 2'-methoxy; note (original language) = 2'-甲氧基修饰
  modified_base 1..3: mod_base = OTHER; note = two adiacentnucleosides a linked by phosphorothioate diestei groups; note (original language) = 相邻的两个核苷之间通过硫代磷酸二酯基连接
  modified_base 19..21: mod_base = OTHER; note = two adiacentnucleosides a linked by phosphorothioate diestei groups; note (original language) = 相邻的两个核苷之间通过硫代磷酸二酯基连接
  modified_base 21: mod_base = OTHER; note = conjugated to A01''; note (original language) = 和A01''缀合
cctcctgttgctgagtatcaa

SEQ ID NO: 23 - RNA, 23 nt, synthetic construct
  source 1..23: mol_type = other RNA
  modified_base 2: mod_base = OTHER; note = modified with 2'-Fluoro; note (original language) = 2'-氟修饰
  modified_base 6: mod_base = OTHER; note = modified with 2'-Fluoro; note (original language) = 2'-氟修饰
  modified_base 14: mod_base = OTHER; note = modified with 2'-Fluoro; note (original language) = 2'-氟修饰
  modified_base 16: mod_base = OTHER; note = modified with 2'-Fluoro; note (original language) = 2'-氟修饰
  modified_base 1: mod_base = OTHER; note = modified with 2'-methoxy; note (original language) = 2'-甲氧基修饰
  modified_base 3..5: mod_base = OTHER; note = modified with 2'-methoxy; note (original language) = 2'-甲氧基修饰
  modified_base 7..13: mod_base = OTHER; note = modified with 2'-methoxy; note (original language) = 2'-甲氧基修饰
  modified_base 15: mod_base = OTHER; note = modified with 2'-methoxy; note (original language) = 2'-甲氧基修饰
  modified_base 17..23: mod_base = OTHER; note = modified with 2'-methoxy; note (original language) = 2'-甲氧基修饰
  modified_base 1..3: mod_base = OTHER; note = two adiacentnucleosides a linked by phosphorothioate diestei groups; note (original language) = 相邻的两个核苷之间通过硫代磷酸二酯基连接
  modified_base 21..23: mod_base = OTHER; note = two adiacentnucleosides a linked by phosphorothioate diestei groups; note (original language) = 相邻的两个核苷之间通过硫代磷酸二酯基连接
  modified_base 1: mod_base = OTHER; note = 5'-E-VP; note (original language) = 5'末端为反式-乙烯基磷酸二酯基
ttgatactcagcaacaggaggag

SEQ ID NO: 24 - RNA, 21 nt, synthetic construct
  source 1..21: mol_type = other RNA
  modified_base 9..11: mod_base = OTHER; note = modified with 2'-Fluoro; note (original language) = 2'-氟修饰
  modified_base 1..8: mod_base = OTHER; note = modified with 2'-methoxy; note (original language) = 2'-甲氧基修饰
  modified_base 12..21: mod_base = OTHER; note = modified with 2'-methoxy; note (original language) = 2'-甲氧基修饰
  modified_base 1..3: mod_base = OTHER; note = two adiacentnucleosides a linked by phosphorothioate diestei groups; note (original language) = 相邻的两个核苷之间通过硫代磷酸二酯基连接
  modified_base 19..21: mod_base = OTHER; note = two adiacentnucleosides a linked by phosphorothioate diestei groups; note (original language) = 相邻的两个核苷之间通过硫代磷酸二酯基连接
  modified_base 21: mod_base = OTHER; note = conjugated to A02''; note (original language) = 和A02''缀合
cctcctgttgctgagtatcaa

SEQ ID NO: 25 - RNA, 21 nt, synthetic construct
  source 1..21: mol_type = other RNA
  modified_base 9..11: mod_base = OTHER; note = modified with 2'-Fluoro; note (original language) = 2'-氟修饰
  modified_base 1..8: mod_base = OTHER; note = modified with 2'-methoxy; note (original language) = 2'-甲氧基修饰
  modified_base 12..21: mod_base = OTHER; note = modified with 2'-methoxy; note (original language) = 2'-甲氧基修饰
  modified_base 1..3: mod_base = OTHER; note = two adiacentnucleosides a linked by phosphorothioate diestei groups; note (original language) = 相邻的两个核苷之间通过硫代磷酸二酯基连接
  modified_base 19..21: mod_base = OTHER; note = two adiacentnucleosides a linked by phosphorothioate diestei groups; note (original language) = 相邻的两个核苷之间通过硫代磷酸二酯基连接
  modified_base 21: mod_base = OTHER; note = conjugated to A03''; note (original language) = 和A03''缀合
cctcctgttgctgagtatcaa

SEQ ID NO: 26 - RNA, 21 nt, synthetic construct
  source 1..21: mol_type = other RNA
  modified_base 9..11: mod_base = OTHER; note = modified with 2'-Fluoro; note (original language) = 2'-氟修饰
  modified_base 1..8: mod_base = OTHER; note = modified with 2'-methoxy; note (original language) = 2'-甲氧基修饰
  modified_base 12..21: mod_base = OTHER; note = modified with 2'-methoxy; note (original language) = 2'-甲氧基修饰
  modified_base 1..3: mod_base = OTHER; note = two adiacentnucleosides a linked by phosphorothioate diestei groups; note (original language) = 相邻的两个核苷之间通过硫代磷酸二酯基连接
  modified_base 19..21: mod_base = OTHER; note = two adiacentnucleosides a linked by phosphorothioate diestei groups; note (original language) = 相邻的两个核苷之间通过硫代磷酸二酯基连接
  modified_base 1: mod_base = OTHER; note = conjugated to A04''; note (original language) = 和A04''缀合
cctcctgttgctgagtatcaa

SEQ ID NO: 27 - RNA, 21 nt, synthetic construct
  source 1..21: mol_type = other RNA
  modified_base 9..11: mod_base = OTHER; note = modified with 2'-Fluoro; note (original language) = 2'-氟修饰
  modified_base 1..8: mod_base = OTHER; note = modified with 2'-methoxy; note (original language) = 2'-甲氧基修饰
  modified_base 12..21: mod_base = OTHER; note = modified with 2'-methoxy; note (original language) = 2'-甲氧基修饰
  modified_base 1..3: mod_base = OTHER; note = two adiacentnucleosides a linked by phosphorothioate diestei groups; note (original language) = 相邻的两个核苷之间通过硫代磷酸二酯基连接
  modified_base 19..21: mod_base = OTHER; note = two adiacentnucleosides a linked by phosphorothioate diestei groups; note (original language) = 相邻的两个核苷之间通过硫代磷酸二酯基连接
  modified_base 1: mod_base = OTHER; note = conjugated to A05''; note (original language) = 和A05''缀合
cctcctgttgctgagtatcaa

SEQ ID NO: 28 - DNA, 20 bp, synthetic construct
  source 1..20: PCR_primers = fwd_name:APP, fwd_seq: gacagacagcacaccctaaa,rev_name: APP, rev_seq: cacacggaggtgtgtcataa; mol_type = other DNA
gacagacagcacaccctaaa

SEQ ID NO: 29 - DNA, 20 bp, synthetic construct
  source 1..20: PCR_primers = fwd_name:APP, fwd_seq: gacagacagcacaccctaaa,rev_name: APP, rev_seq: cacacggaggtgtgtcataa; mol_type = other DNA
cacacggaggtgtgtcataa

SEQ ID NO: 30 - DNA, 24 bp, synthetic construct
  source 1..24: mol_type = other DNA
atcccaagaaagccgctcagatcc

SEQ ID NO: 31 - DNA, 22 bp, synthetic construct
  source 1..22: PCR_primers = fwd_name:GAPDH, fwd_seq: ccaggtggtctcctctgacttc,rev_name:GAPDH, rev_seq: gtggtcgttgagggcaatg; mol_type = other DNA
ccaggtggtctcctctgacttc

SEQ ID NO: 32 - DNA, 19 bp, synthetic construct
  source 1..19: PCR_primers = fwd_name:GAPDH, fwd_seq: ccaggtggtctcctctgacttc,rev_name:GAPDH, rev_seq: gtggtcgttgagggcaatg; mol_type = other DNA
gtggtcgttgagggcaatg

SEQ ID NO: 33 - DNA, 25 bp, synthetic construct
  source 1..25: mol_type = other DNA
acagcgacacccactcctccacctt

SEQ ID NO: 34 - DNA, 20 bp, synthetic construct
  source 1..20: PCR_primers = fwd_name:miceAPP, fwd_seq: tgacaagaaggccgttatcc,rev_name: miceAPP, rev_seq: ggccatgtgtgtctctacaa; mol_type = other DNA
tgacaagaaggccgttatcc

SEQ ID NO: 35 - DNA, 20 bp, synthetic construct
  source 1..20: PCR_primers = fwd_name:miceAPP, fwd_seq: tgacaagaaggccgttatcc,rev_name: miceAPP, rev_seq: ggccatgtgtgtctctacaa; mol_type = other DNA
ggccatgtgtgtctctacaa

SEQ ID NO: 36 - DNA, 27 bp, synthetic construct
  source 1..27: mol_type = other DNA
ctgtctctcattggctgcttcctgttc

SEQ ID NO: 37 - DNA, 23 bp, synthetic construct
  source 1..23: PCR_primers = fwd_name:MAPT, fwd_seq: ctctcaggtttgtggaggtaatc,rev_name: MAPT, rev_seq: ccagggttcttaggaggtatttg; mol_type = other DNA
ctctcaggtttgtggaggtaatc

SEQ ID NO: 38 - DNA, 23 bp, synthetic construct
  source 1..23: PCR_primers = fwd_name:MAPT, fwd_seq: ctctcaggtttgtggaggtaatc,rev_name: MAPT, rev_seq: ccagggttcttaggaggtatttg; mol_type = other DNA
ccagggttcttaggaggtatttg

SEQ ID NO: 39 - DNA, 27 bp, synthetic construct
  source 1..27: mol_type = other DNA
cttctcttcctgctgccttcttgtgat

SEQ ID NO: 40 - DNA, 20 bp, synthetic construct
  source 1..20: PCR_primers = fwd_name:mGAPDH, fwd_seq: aacagcaactcccactcttc,rev_name: mGAPDH, rev_seq: cctgttgctgtagccgtatt; mol_type = other DNA
aacagcaactcccactcttc

SEQ ID NO: 41 - DNA, 20 bp, synthetic construct
  source 1..20: PCR_primers = fwd_name:mGAPDH, fwd_seq: aacagcaactcccactcttc,rev_name: mGAPDH, rev_seq: cctgttgctgtagccgtatt; mol_type = other DNA
cctgttgctgtagccgtatt

SEQ ID NO: 42 - DNA, 27 bp, synthetic construct
  source 1..27: mol_type = other DNA
aaagttgtcattgagagcaatgccagc

SEQ ID NO: 43 - DNA, 22 bp, synthetic construct
  source 1..22: PCR_primers = fwd_name:pmp22, fwd_seq: gtggcatctcaactcggattac,rev_name: pmp22, rev_seq: cgtttccgcaagatcacataga; mol_type = other DNA
gtggcatctcaactcggattac

SEQ ID NO: 44 - DNA, 22 bp, synthetic construct
  source 1..22: PCR_primers = fwd_name:pmp22, fwd_seq: gtggcatctcaactcggattac,rev_name: pmp22, rev_seq: cgtttccgcaagatcacataga; mol_type = other DNA
cgtttccgcaagatcacataga

SEQ ID NO: 45 - DNA, 24 bp, synthetic construct
  source 1..24: mol_type = other DNA
ctacggtttcgcctacatcctggc

SEQ ID NO: 46 - DNA, 20 bp, synthetic construct
  source 1..20: PCR_primers = fwd_name:sarm1, fwd_seq: ctttaagctgcggcaagaac,rev_name: sarm1, rev_seq: attcgtgggaccacttgatac; mol_type = other DNA
ctttaagctgcggcaagaac

SEQ ID NO: 47 - DNA, 21 bp, synthetic construct
  source 1..21: PCR_primers = fwd_name:sarm1, fwd_seq: ctttaagctgcggcaagaac,rev_name: sarm1, rev_seq: attcgtgggaccacttgatac; mol_type = other DNA
attcgtgggaccacttgatac

SEQ ID NO: 48 - DNA, 26 bp, synthetic construct
  source 1..26: mol_type = other DNA
catgcaggctgtgcttactttcaacg